European Patent Specification EP 3 791 856 B1, published June 18, 2025. Title: TOOTHPASTE COMPOSITION FOR ALLEVIATING DENTINE HYPERESTHESIA. Applicant: HysensBio. The sequence listing filed with the application follows.

SEQUENCE LISTING (104 sequences)

SEQ ID NO: 1 - protein, 10 aa, Artificial Sequence
  Novel peptide
KYQRRKKNKY

SEQ ID NO: 2 - protein, 10 aa, Artificial Sequence
  Novel peptide
KYQRRKRNKY

SEQ ID NO: 3 - protein, 10 aa, Artificial Sequence
  Novel peptide
KYQRRRKNKY

SEQ ID NO: 4 - protein, 10 aa, Artificial Sequence
  Novel peptide
KYQRRRRNKY

SEQ ID NO: 5 - protein, 10 aa, Artificial Sequence
  Novel peptide
KYQRKKKNKY

SEQ ID NO: 6 - protein, 10 aa, Artificial Sequence
  Novel peptide
KYQRKRKNKY

SEQ ID NO: 7 - protein, 10 aa, Artificial Sequence
  Novel peptide
KYQRKKRNKY

SEQ ID NO: 8 - protein, 10 aa, Artificial Sequence
  Novel peptide
KYQRKRRNKY

SEQ ID NO: 9 - protein, 10 aa, Artificial Sequence
  Novel peptide
KYQRRKKSKY

SEQ ID NO: 10 - protein, 10 aa, Artificial Sequence
  Novel peptide
KYQRRKRSKY

SEQ ID NO: 11 - protein, 10 aa, Artificial Sequence
  Novel peptide
KYQRRRKSKY

SEQ ID NO: 12 - protein, 10 aa, Artificial Sequence
  Novel peptide
KYQRRRRSKY

SEQ ID NO: 13 - protein, 10 aa, Artificial Sequence
  Novel peptide
KYQRKKKSKY

SEQ ID NO: 14 - protein, 10 aa, Artificial Sequence
  Novel peptide
KYQRKRKSKY

SEQ ID NO: 15 - protein, 10 aa, Artificial Sequence
  Novel peptide
KYQRKKRSKY

SEQ ID NO: 16 - protein, 10 aa, Artificial Sequence
  Novel peptide
KYQRKRRSKY

SEQ ID NO: 17 - protein, 10 aa, Artificial Sequence
  Novel peptide
KYQRRKKNYK

SEQ ID NO: 18 - protein, 10 aa, Artificial Sequence
  Novel peptide
KYQRRKRNYK

SEQ ID NO: 19 - protein, 10 aa, Artificial Sequence
  Novel peptide
KYQRRRKNYK

SEQ ID NO: 20 - protein, 10 aa, Artificial Sequence
  Novel peptide
KYQRRRRNYK

SEQ ID NO: 21 - protein, 10 aa, Artificial Sequence
  Novel peptide
KYQRKKKNYK

SEQ ID NO: 22 - protein, 10 aa, Artificial Sequence
  Novel peptide
KYQRKRKNYK

SEQ ID NO: 23 - protein, 10 aa, Artificial Sequence
  Novel peptide
KYQRKKRNYK

SEQ ID NO: 24 - protein, 10 aa, Artificial Sequence
  Novel peptide
KYQRKRRNYK

SEQ ID NO: 25 - protein, 10 aa, Artificial Sequence
  Novel peptide
KYQRRKKSYK

SEQ ID NO: 26 - protein, 10 aa, Artificial Sequence
  Novel peptide
KYQRRKRSYK

SEQ ID NO: 27 - protein, 10 aa, Artificial Sequence
  Novel peptide
KYQRRRKSYK

SEQ ID NO: 28 - protein, 10 aa, Artificial Sequence
  Novel peptide
KYQRRRRSYK

SEQ ID NO: 29 - protein, 10 aa, Artificial Sequence
  Novel peptide
KYQRKKKSYK

SEQ ID NO: 30 - protein, 10 aa, Artificial Sequence
  Novel peptide
KYQRKRKSYK

SEQ ID NO: 31 - protein, 10 aa, Artificial Sequence
  Novel peptide
KYQRKKRSYK

SEQ ID NO: 32 - protein, 10 aa, Artificial Sequence
  Novel peptide
KYQRKRRSYK

SEQ ID NO: 33 - protein, 10 aa, Artificial Sequence
  Novel peptide
KYRQRKKNKY

SEQ ID NO: 34 - protein, 10 aa, Artificial Sequence
  Novel peptide
KYRQRKRNKY

SEQ ID NO: 35 - protein, 10 aa, Artificial Sequence
  Novel peptide
KYRQRRKNKY

SEQ ID NO: 36 - protein, 10 aa, Artificial Sequence
  Novel peptide
KYRQRRRNKY

SEQ ID NO: 37 - protein, 10 aa, Artificial Sequence
  Novel peptide
KYRQKKKNKY

SEQ ID NO: 38 - protein, 10 aa, Artificial Sequence
  Novel peptide
KYRQKRKNKY

SEQ ID NO: 39 - protein, 10 aa, Artificial Sequence
  Novel peptide
KYRQKKRNKY

SEQ ID NO: 40 - protein, 10 aa, Artificial Sequence
  Novel peptide
KYRQKRRNKY

SEQ ID NO: 41 - protein, 10 aa, Artificial Sequence
  Novel peptide
KYRQRKKSKY

SEQ ID NO: 42 - protein, 10 aa, Artificial Sequence
  Novel peptide
KYRQRKRSKY

SEQ ID NO: 43 - protein, 10 aa, Artificial Sequence
  Novel peptide
KYRQRRKSKY

SEQ ID NO: 44 - protein, 10 aa, Artificial Sequence
  Novel peptide
KYRQRRRSKY

SEQ ID NO: 45 - protein, 10 aa, Artificial Sequence
  Novel peptide
KYRQKKKSKY

SEQ ID NO: 46 - protein, 10 aa, Artificial Sequence
  Novel peptide
KYRQKRKSKY

SEQ ID NO: 47 - protein, 10 aa, Artificial Sequence
  Novel peptide
KYRQKKRSKY

SEQ ID NO: 48 - protein, 10 aa, Artificial Sequence
  Novel peptide
KYRQKRRSKY

SEQ ID NO: 49 - protein, 10 aa, Artificial Sequence
  Novel peptide
KYRQRKKNYK

SEQ ID NO: 50 - protein, 10 aa, Artificial Sequence
  Novel peptide
KYRQRKRNYK

SEQ ID NO: 51 - protein, 10 aa, Artificial Sequence
  Novel peptide
KYRQRRKNYK

SEQ ID NO: 52 - protein, 10 aa, Artificial Sequence
  Novel peptide
KYRQRRRNYK

SEQ ID NO: 53 - protein, 10 aa, Artificial Sequence
  Novel peptide
KYRQKKKNYK

SEQ ID NO: 54 - protein, 10 aa, Artificial Sequence
  Novel peptide
KYRQKRKNYK

SEQ ID NO: 55 - protein, 10 aa, Artificial Sequence
  Novel peptide
KYRQKKRNYK

SEQ ID NO: 56 - protein, 10 aa, Artificial Sequence
  Novel peptide
KYRQKRRNYK

SEQ ID NO: 57 - protein, 10 aa, Artificial Sequence
  Novel peptide
KYRQRKKSYK

SEQ ID NO: 58 - protein, 10 aa, Artificial Sequence
  Novel peptide
KYRQRKRSYK

SEQ ID NO: 59 - protein, 10 aa, Artificial Sequence
  Novel peptide
KYRQRRKSYK

SEQ ID NO: 60 - protein, 10 aa, Artificial Sequence
  Novel peptide
KYRQRRRSYK

SEQ ID NO: 61 - protein, 10 aa, Artificial Sequence
  Novel peptide
KYRQKKKSYK

SEQ ID NO: 62 - protein, 10 aa, Artificial Sequence
  Novel peptide
KYRQKRKSYK

SEQ ID NO: 63 - protein, 10 aa, Artificial Sequence
  Novel peptide
KYRQKKRSYK

SEQ ID NO: 64 - protein, 10 aa, Artificial Sequence
  Novel peptide
KYRQKRRSYK

SEQ ID NO: 65 - protein, 10 aa, Artificial Sequence
  Novel peptide
KYKQRKKNKY

SEQ ID NO: 66 - protein, 10 aa, Artificial Sequence
  Novel peptide
KYKQRKRNKY

SEQ ID NO: 67 - protein, 10 aa, Artificial Sequence
  Novel peptide
KYKQRRKNKY

SEQ ID NO: 68 - protein, 10 aa, Artificial Sequence
  Novel peptide
KYKQRRRNKY

SEQ ID NO: 69 - protein, 10 aa, Artificial Sequence
  Novel peptide
KYKQKKKNKY

SEQ ID NO: 70 - protein, 10 aa, Artificial Sequence
  Novel peptide
KYKQKRKNKY

SEQ ID NO: 71 - protein, 10 aa, Artificial Sequence
  Novel peptide
KYKQKKRNKY

SEQ ID NO: 72 - protein, 10 aa, Artificial Sequence
  Novel peptide
KYKQKRRNKY

SEQ ID NO: 73 - protein, 10 aa, Artificial Sequence
  Novel peptide
KYKQRKKSKY

SEQ ID NO: 74 - protein, 10 aa, Artificial Sequence
  Novel peptide
KYKQRKRSKY

SEQ ID NO: 75 - protein, 10 aa, Artificial Sequence
  Novel peptide
KYKQRRKSKY

SEQ ID NO: 76 - protein, 10 aa, Artificial Sequence
  Novel peptide
KYKQRRRSKY

SEQ ID NO: 77 - protein, 10 aa, Artificial Sequence
  Novel peptide
KYKQKKKSKY

SEQ ID NO: 78 - protein, 10 aa, Artificial Sequence
  Novel peptide
KYKQKRKSKY

SEQ ID NO: 79 - protein, 10 aa, Artificial Sequence
  Novel peptide
KYKQKKRSKY

SEQ ID NO: 80 - protein, 10 aa, Artificial Sequence
  Novel peptide
KYKQKRRSKY

SEQ ID NO: 81 - protein, 10 aa, Artificial Sequence
  Novel peptide
KYKQRKKNYK

SEQ ID NO: 82 - protein, 10 aa, Artificial Sequence
  Novel peptide
KYKQRKRNYK

SEQ ID NO: 83 - protein, 10 aa, Artificial Sequence
  Novel peptide
KYKQRRKNYK

SEQ ID NO: 84 - protein, 10 aa, Artificial Sequence
  Novel peptide
KYKQRRRNYK

SEQ ID NO: 85 - protein, 10 aa, Artificial Sequence
  Novel peptide
KYKQKKKNYK

SEQ ID NO: 86 - protein, 10 aa, Artificial Sequence
  Novel peptide
KYKQKRKNYK

SEQ ID NO: 87 - protein, 10 aa, Artificial Sequence
  Novel peptide
KYKQKKRNYK

SEQ ID NO: 88 - protein, 10 aa, Artificial Sequence
  Novel peptide
KYKQKRRNYK

SEQ ID NO: 89 - protein, 10 aa, Artificial Sequence
  Novel peptide
KYKQRKKSYK

SEQ ID NO: 90 - protein, 10 aa, Artificial Sequence
  Novel peptide
KYKQRKRSYK

SEQ ID NO: 91 - protein, 10 aa, Artificial Sequence
  Novel peptide
KYKQRRKSYK

SEQ ID NO: 92 - protein, 10 aa, Artificial Sequence
  Novel peptide
KYKQRRRSYK

SEQ ID NO: 93 - protein, 10 aa, Artificial Sequence
  Novel peptide
KYKQKKKSYK

SEQ ID NO: 94 - protein, 10 aa, Artificial Sequence
  Novel peptide
KYKQKRKSYK

SEQ ID NO: 95 - protein, 10 aa, Artificial Sequence
  Novel peptide
KYKQKKRSYK

SEQ ID NO: 96 - protein, 10 aa, Artificial Sequence
  Novel peptide
KYKQKRRSYK

SEQ ID NO: 97 - DNA, 21 bp, Artificial Sequence
  primer
attccggttccccagttagta

SEQ ID NO: 98 - DNA, 20 bp, Artificial Sequence
  primer
ctgttgctagtggtgctgtt

SEQ ID NO: 99 - DNA, 21 bp, Artificial Sequence
  primer
aggtcggtgtgaacggatttg

SEQ ID NO: 100 - DNA, 23 bp, Artificial Sequence
  primer
tgtagaccatgtagttgaggtca

SEQ ID NO: 101 - DNA, 23 bp, Artificial Sequence
  primer
cattctccttgtgttcctttggg

SEQ ID NO: 102 - DNA, 21 bp, Artificial Sequence
  primer
tgtggtcactatttgcctgtg

SEQ ID NO: 103 - DNA, 19 bp, Artificial Sequence
  primer
ccctgaagtcgaggagctg

SEQ ID NO: 104 - DNA, 19 bp, Artificial Sequence
  primer
ctgctgcacctctaagcga